European Patent Application EP 4 190 350 A1, published June 7, 2023. Title: FILOVIRUS CONSENSUS ANTIGENS, NUCLEIC ACID CONSTRUCTS AND VACCINES MADE THEREFROM, AND METHODS OF USING THE SAME. Applicant: The Trustees of the University of Pennsylvania. The sequence listing filed with the application follows.

SEQUENCE LISTING (66 sequences)

SEQ ID NO: 1 - protein, 676 aa, synthetic construct
MGVTGILQLPRDRFKRTSFFLWVIILFQRTFSIPLGVIHNSTLQVSDVDKLVCRDKLSSTNQLRSVGLNLEGNGVATDVPSATKRWGFRSGVPPKVVNYEAGEWAENCYNLEIKKPDGSECLPAAPDGIRGFPRCRYVHKVSGTGPCAGDFAFHKEGAFFLYDRLASTVIYRGTTFAEGVVAFLILPQAKKDFFSSHPLREPVNATEDPSSGYYSTTIRYQATGFGTNETEYLFEVDNLTYVQLESRFTPQFLLQLNETIYTSGKRSNTTGKLIWKVNPEIDTTIGEWAFWETKKNLTRKIRSEELSFTAVSNRAKNISGQSPARTSSDPGTNTTTEDHKIMASENSSAMVQVHSQGREAAVSHLTTLATISTSPQSPTTKPGPDNSTHNTPVYKLDISEATQVEQHHRRTDNDSTASDTPPATTAAGPPKAENTNTSKSTDLLDPATTTSPQNHSETAGNNNTHHQDTGEESASSGKLGLITNTIAGVAGLITGGRRTRREAIVNAQPKCNPNLHYWTTQDEGAAIGLAWIPYFGPAAEGIYTEGLMHNQDGLICGLRQLANETTQALQLFLRATTELRTFSILNRKAIDFLLQRWGGTCHILGPDCCIEPHDWTKNITDKIDQIIHDFVDKTLPDQGDNDNWWTGWRQWIPAGIGVTGVIIAVIALFCICKFVF

SEQ ID NO: 2 - protein, 676 aa, synthetic construct
MEGLSLLQLPRDKFRKSSFFVWVIILFQKAFSMPLGVVTNSTLEVTEIDQLVCKDHLASTDQLKSVGLNLEGSGVSTDIPSATKRWGFRSGVPPKVVSYEAGEWAENCYNLEIKKPDGSECLPPPPDGVRGFPRCRYVHKAQGTGPCPGDYAFHKDGAFFLYDRLASTVIYRGVNFAEGVIAFLILAKPKETFLQSPPIREAVNYTENTSSYYATSYLEYEIENFGAQHSTTLFKINNNTFVLLDRPHTPQFLFQLNDTIHLHQQLSNTTGKLIWTLDANINADIGEWAFWENKKNLSEQLRGEELSFETLSLNETEDDDATSSRTTKGRISDRATRKYSDLVPKDSPGMVSLHVPEGETTLPSQNSTEGRRVDVNTQETITETTATIIGTNGNNMQISTIGTGLSSSQILSSSPTMAPSPETQTSTTYTPKLPVMTTEEPTTPPRNSPGSTTEAPTLTTPENITTAVKTVLPQESTSNGLITSTVTGILGSLGLRKRSRRQVNTRATGKCNPNLHYWTAQEQHNAAGIAWIPYFGPGAEGIYTEGLMHNQNALVCGLRQLANETTQALQLFLRATTELRTYTILNRKAIDFLLRRWGGTCRILGPDCCIEPHDWTKNITDKINQIIHDFIDNPLPNQDNDDNWWTGWRQWIPAGIGITGIIIAIIALLCVCKLLC

SEQ ID NO: 3 - protein, 681 aa, Marburg marburgvirus
MKTTCLLISLILIQGVKTLPILEIASNIQPQNVDSVCSGTLQKTEDVHLMGFTLSGQKVADSPLEASKRWAFRAGVPPKNVEYTEGEEAKTCYNISVTDPSGKSLLLDPPTNIRDYPKCKTIHHIQGQNPHAQGIALHLWGAFFLYDRIASTTMYRGKVFTEGNIAAMIVNKTVHKMIFSRQGQGYRHMNLTSTNKYWTSSNGTQTNDTGCFGTLQEYNSTKNQTCAPSKKPLPLPTAHPEVKLTSTSTDATKLNTTDPNSDDEDLTTSGSGSGEQEPYTTSDAATKQGLSSTMPPTPSPQPSTPQQGGNNTNHSQGVVTEPGKTNTTAQPSMPPHNTTTISTNNTSKHNLSTPSVPIQNATNYNTQSTAPENEQTSAPSKTTLLPTENPTTAKSTNSTKSPTTTVPNTTNKYSTSPSPTPNSTAQHLVYFRRKRNILWREGDMFPFLDGLINAPIDFDPVPNTKTIFDESSSSGASAEEDQHASPNISLTLSYFPKVNENTAHSGENENDCDAELRIWSVQEDDLAAGLSWIPFFGPGIEGLYTAGLIKNQNNLVCRLRRLANQTAKSLELLLRVTTEERTFSLINRHAIDFLLARWGGTCKVLGPDCCIGIEDLSRNISEQIDQIKKDEQKEGTGWGLGGKWWTSDWGVLTNLGILLLLSIAVLIALSCICRIFTKYIG

SEQ ID NO: 4 - protein, 681 aa, synthetic construct
MKTIYFLISLILIQSIKTLPVLEIASNSQPQDVDSVCSGTLQKTEDVHLMGFTLSGQKVADSPLEASKRWAFRTGVPPKNVEYTEGEEAKTCYNISVTDPSGKSLLLDPPSNIRDYPKCKTVHHIQGQNPHAQGIALHLWGAFFLYDRVASTTMYRGKVFTEGNIAAMIVNKTVHRMIFSRQGQGYRHMNLTSTNKYWTSSNETRRNDTGCFGILQEYNSTNNQTCSPSLKPPSLPTVTPSIHSTNTQINTAKSGTMNPSSDDEDLMISGSGSGEQGPHTTLNVVTEQKQSSTILSTPSLHPSTSQHEQNSTNPSRHAVTEHNGTDPTTQPATLLNNTNTTPTYNTLKYNLSTPSPPTRNITNNDTQRELAESEQTNAQLNTTLDPTENPTTAQDTNSTTNIIMTTSDITSKHPTNSSPDSSPTTRPPIYFRKKRSIFWKEGDIFPFLDGLINTEIDFDPIPNTETIFDESPSFNTSTNEEQHTPPNISLTFSYFPDKNGDTAYSGENENDCDAELRIWSVQEDDLAAGLSWIPFFGPGIEGLYTAGLIKNQNNLVCRLRRLANQTAKSLELLLRVTTEERTFSLINRHAIDFLLTRWGGTCKVLGPDCCIGIEDLSKNISEQIDKIRKDEQKEETGWGLGGKWWTSDWGVLTNLGILLLLSIAVLIALSCICRIFTKYIG

SEQ ID NO: 5 - protein, 681 aa, synthetic construct
MRTTCFFISLILIQGIKTLPILEIASNDQPQNVDSVCSGTLQKTEDVHLMGFTLSGQKVADSPLEASKRWAFRTGVPPKNVEYTEGEEAKTCYNISVTDPSGKSLLLDPPTNVRDYPKCKTIHHIQGQNPHAQGIALHLWGAFFLYDRIASTTMYRGKVFTEGNIAAMIVNKTVHKMIFSRQGQGYRHMNLTSTNKYWTSSNGTQTNDTGCFGTLQEYNSTKNQTCAPSKTPPPPPTARPEIKPTSTPTDATRLNTTNPNSDDEDLTTSGSGSGEQEPYTTSDAVTKQGLSSTMPPTPSPQPGTPQQGGNNTNHSQDAATELDNTNTTAQPPTPSHNTTTISTNNTSKHNLSTLSEPPQNTTNPNTQSMATENEKTSAPPKTTLPPTESPTTEKSTNNTKSPTTMEPNTTNGHFTSPSSTPNSTTQHLIYFRRKRSILWREGDMFPFLDGLINAPIDFDPVPNTKTIFDESSSSGASAEEDQHASSNISLTLSYLPHTSENTAYSGENENDCDAELRIWSVQEDDLAAGLSWIPFFGPGIEGLYTAGLIKNQNNLVCRLRRLANQTAKSLELLLRVTTEERTFSLINRHAIDFLLTRWGGTCKVLGPDCCIGIEDLSRNISEQIDQIKKDEQKEGTGWGLGGKWWTSDWGVLTNLGILLLLSIAVLIALSCICRIFTKYIG

SEQ ID NO: 6 - protein, 681 aa, synthetic construct
MKTTCLFISLILIQGIKTLPILEIASNNQPQNVDSVCSGTLQKTEDVHLMGFTLSGQKVADSPLEASKRWAFRTGVPPKNVEYTEGEEAKTCYNISVTDPSGKSLLLDPPTNIRDYPKCKTIHHIQGQNPHAQGIALHLWGAFFLYDRIASTTMYRGRVFTEGNIAAMIVNKTVHKMIFSRQGQGYRHMNLTSTNKYWTSNNGTQTNDTGCFGALQEYNSTKNQTCAPSKIPSPLPTARPEIKPTSTPTDATKLNTTDPNSDDEDLATSGSGSGEQEPHTTSDAVTKQGLSSTMPPTPSPQPSTPQQEGNNTDHSQDAVTEPNKTNTTAQPSMPPHNTTAISTNNTSKHNFSTLSAPLQNTTNYDTQSTATENEQTSAPSKTTLPPTGNLTTAKSTNNTKGPTTTAPNMTNGHLTSPSPTPNPTTQHLVYFRKKRSILWREGDMFPFLDGLINAPIDFDPVPNTKTIFDESSSSGASAEEDQHASPNISLTLSYFPNINENTAYSGENENDCDAELRIWSVQEDDLAAGLSWIPFFGPGIEGLYTAGLIKNQNNLVCRLRRLANQTAKSLELLLRVTTEERTFSLINRHAIDFLLTRWGGTCKVLGPDCCIGIEDLSRNISEQIDQIKKDEQKEGTGWGLGGKWWTSDWGVLTNLGILLLLSIAVLIALSCICRIFTKYIG

SEQ ID NO: 7 - protein, 15 aa, Marburg marburgvirus
IQGVKTLPILEIASN

SEQ ID NO: 8 - protein, 15 aa, Marburg marburgvirus
ASNIQPQNVDSVCSG

SEQ ID NO: 9 - protein, 15 aa, Marburg marburgvirus
SKRWAFRAGVPPKNV

SEQ ID NO: 10 - protein, 15 aa, Marburg marburgvirus
GKVFTEGNIAAMIVN

SEQ ID NO: 11 - protein, 15 aa, Marburg marburgvirus
GNIAAMIVNKTVHKM

SEQ ID NO: 12 - protein, 15 aa, Marburg marburgvirus
GNIAAMIVNKTVHKM

SEQ ID NO: 13 - protein, 15 aa, Marburg marburgvirus
IVNKTVHKMIFSRQG

SEQ ID NO: 14 - protein, 15 aa, Marburg marburgvirus
HKMIFSRQGQGYRHM

SEQ ID NO: 15 - protein, 15 aa, Marburg marburgvirus
RQGQGYRHMNLTSTN

SEQ ID NO: 16 - protein, 15 aa, Marburg marburgvirus
RHMNLTSTNKYWTSS

SEQ ID NO: 17 - protein, 15 aa, Marburg marburgvirus
LPTENPTTAKSTNST

SEQ ID NO: 18 - protein, 15 aa, Marburg marburgvirus
PNSTAQHLVYFRRKR

SEQ ID NO: 19 - protein, 15 aa, Marburg marburgvirus
HLVYFRRKRNILWRE

SEQ ID NO: 20 - protein, 15 aa, Marburg marburgvirus
GLSWIPFFGPGIEGL

SEQ ID NO: 21 - protein, 15 aa, Marburg marburgvirus
GLIKNQNNLVCRLRR

SEQ ID NO: 22 - protein, 15 aa, Marburg marburgvirus
NNLVCRLRRLANQTA

SEQ ID NO: 23 - protein, 15 aa, Marburg marburgvirus
TTEERTFSLINRHAI

SEQ ID NO: 24 - protein, 15 aa, Marburg marburgvirus
HAIDFLLARWGGTCK

SEQ ID NO: 25 - protein, 15 aa, Marburg marburgvirus
TCKVLGPDCCIGIED

SEQ ID NO: 26 - protein, 15 aa, synthetic construct
FFVWVIILFQKAFSM

SEQ ID NO: 27 - protein, 15 aa, synthetic construct
RWGFRSGVPPKVVSY

SEQ ID NO: 28 - protein, 15 aa, synthetic construct
YNLEIKKPDGSECLP

SEQ ID NO: 29 - protein, 15 aa, synthetic construct
HKAQGTGPCPGDYAF

SEQ ID NO: 30 - protein, 15 aa, synthetic construct
GAFFLYDRLASTVIY

SEQ ID NO: 31 - protein, 15 aa, synthetic construct
NFAEGVIAFLILAKP

SEQ ID NO: 32 - protein, 15 aa, synthetic construct
SYYATSYLEYEIENF

SEQ ID NO: 33 - protein, 15 aa, synthetic construct
FVLLDRPHTPQFLFQ

SEQ ID NO: 34 - protein, 15 aa, synthetic construct
NITTAVKTVLPQEST

SEQ ID NO: 35 - protein, 15 aa, synthetic construct
TGILGSLGLRKRSRR

SEQ ID NO: 36 - protein, 15 aa, synthetic construct
LGLRKRSRRQVNTRA

SEQ ID NO: 37 - protein, 15 aa, synthetic construct
IAWIPYFGPGAEGIY

SEQ ID NO: 38 - protein, 15 aa, synthetic construct
TELRTYTILNRKAID

SEQ ID NO: 39 - protein, 15 aa, synthetic construct
CRILGPDCCIEPHDW

SEQ ID NO: 40 - protein, 15 aa, synthetic construct
QIIHDFIDNPLPNQD

SEQ ID NO: 41 - protein, 15 aa, synthetic construct
GIGITGIIIAIIALL

SEQ ID NO: 42 - protein, 15 aa, synthetic construct
FSIPLGVIHNSTLQV

SEQ ID NO: 43 - protein, 15 aa, synthetic construct
RWGFRSGVPPKVVNY

SEQ ID NO: 44 - protein, 15 aa, synthetic construct
YNLEIKKPDGSECLP

SEQ ID NO: 45 - protein, 15 aa, synthetic construct
GAFFLYDRLASTVIY

SEQ ID NO: 46 - protein, 15 aa, synthetic construct
GAFFLYDRLASTVIY

SEQ ID NO: 47 - protein, 15 aa, synthetic construct
TFAEGVVAFLILPQA

SEQ ID NO: 48 - protein, 15 aa, synthetic construct
PQAKKDFFSSHPLRE

SEQ ID NO: 49 - protein, 15 aa, synthetic construct
FFSSHPLREPVNATE

SEQ ID NO: 50 - protein, 15 aa, synthetic construct
EVDNLTYVQLESRFT

SEQ ID NO: 51 - protein, 15 aa, synthetic construct
YVQLESRFTPQFLLQ

SEQ ID NO: 52 - protein, 15 aa, synthetic construct
TTIGEWAFWETKKNL

SEQ ID NO: 53 - protein, 15 aa, synthetic construct
AFWETKKNLTRKIRS

SEQ ID NO: 54 - protein, 15 aa, synthetic construct
KNLTRKIRSEELSFT

SEQ ID NO: 55 - protein, 15 aa, synthetic construct
SQGREAAVSHLTTLA

SEQ ID NO: 56 - protein, 15 aa, synthetic construct
DNSTHNTPVYKLDIS

SEQ ID NO: 57 - protein, 15 aa, synthetic construct
TPVYKLDISEATQVE

SEQ ID NO: 58 - protein, 15 aa, synthetic construct
PPATTAAGPPKAENT

SEQ ID NO: 59 - protein, 15 aa, synthetic construct
TRREAIVNAQPKCNP

SEQ ID NO: 60 - protein, 15 aa, synthetic construct
LAWIPYFGPAAEGIY

SEQ ID NO: 61 - protein, 15 aa, synthetic construct
TELRTFSILNRKAID

SEQ ID NO: 62 - protein, 15 aa, synthetic construct
CHILGPDCCIEPHDW

SEQ ID NO: 63 - protein, 15 aa, Homo sapiens
CHILGPDCCIEPHDW

SEQ ID NO: 64 - DNA, 2034 bp, synthetic construct
  source 1..2034: mol_type = other DNA
atgggggtcactgggattctgcagctgcctagagatcgcttcaagcgaacctctttctttctgtgggtcatcattctgttccagaggacttttagtatccctctgggcgtcattcacaattctaccctgcaggtgagtgacgtcgataagctggtgtgtcgggacaaactgagctccaccaaccagctgagatctgtcggcctgaatctggaggggaacggagtggctaccgatgtcccaagtgcaacaaagagatgggggtttcgctcaggagtgccccctaaagtggtcaattacgaggccggggaatgggctgagaattgctataacctggaaatcaagaaacccgacggatcagagtgtctgccagccgctcccgatgggattcgcggattccctagatgcagatacgtgcacaaggtcagcggcaccgggccatgtgcaggagacttcgcctttcataaagaaggcgccttctttctgtacgatagactggcttccaccgtgatctatagggggaccacattcgccgagggagtggtcgcttttctgattctgcctcaggccaagaaagacttcttttctagtcatcctctgcgggaaccagtgaacgctaccgaggaccccagcagcggctactattccactaccatcagataccaggccacaggattcggcaccaatgagacagaatacctgtttgaagtggacaacctgacatatgtccagctggagtctaggttcactccccagtttctgctgcagctgaatgaaactatctataccagtggcaagcgctcaaatacaactgggaagctgatttggaaagtgaaccctgagatcgataccacaattggcgaatgggccttttgggagaccaagaaaaacctgacacggaagatcagaagcgaggaactgtccttcaccgcagtgagtaatagggccaaaaacatttcaggccagagcccagcacgaacttcctctgaccccgggaccaatactaccacagaagatcacaagatcatggccagcgagaacagttcagctatggtgcaggtccactcccagggaagggaggcagccgtgtctcatctgactaccctggccacaatctctactagtccccagagccccacaactaagcccgggcctgacaatagcacccataacacacctgtgtacaaactggatatctccgaagccacccaggtcgagcagcaccatcggagaacagacaatgattccactgcatctgacacccctccagcaaccacagctgcaggaccccccaaggctgagaatactaacaccagcaaaagcaccgacctgctggaccccgcaactaccacatcaccacagaaccacagcgagacagccgggaacaataacactcaccatcaggacaccggagaggaatccgccagctccggcaagctggggctgatcacaaatactattgctggagtggcaggactgatcacaggcgggaggcgaactcgacgagaagctattgtgaacgcacagcccaaatgcaatcctaacctgcactattggactacccaggacgagggagcagctatcggactggcatggattccatactttgggcccgcagccgaaggaatctataccgagggcctgatgcataatcaggatggactgatctgtggcctgcggcagctggctaacgaaacaactcaggcactgcagctgttcctgcgagctaccacagagctgcggacctttagcatcctgaatcgcaaggcaattgacttcctgctgcagcgatggggaggcacatgccacatcctgggaccagactgctgtattgagcctcatgattggacaaagaacatcactgacaaaattgatcagatcattcacgacttcgtggataaaacactgccagatcagggggacaatgataactggtggactggatggagacagtggattcccgccggcattggcgtcaccggcgtcattattgccgtcattgctctgttctgtatttgtaagttcgtgttctgataa

SEQ ID NO: 65 - DNA, 2034 bp, synthetic construct
  source 1..2034: mol_type = other DNA
atggagggactgtcactgctgcagctgcctagagataagttcaggaaaagctccttctttgtgtgggtcatcattctgttccagaaggccttttcaatgcccctgggcgtggtcactaatagcaccctggaagtgacagagatcgatcagctggtctgtaaggaccacctggcttcaactgatcagctgaaaagcgtggggctgaacctggagggatcaggcgtcagcactgatattccttctgcaaccaagagatggggatttcgcagcggagtgccccctaaagtggtctcctacgaagcaggggagtgggccgaaaattgctataacctggagatcaagaaaccagatggcagcgaatgtctgccaccccctccagacggggtgcgcggattccccagatgcagatacgtccacaaggcccaggggaccggaccttgtccaggagactatgcctttcataaagatggcgctttctttctgtacgaccgcctggctagtacagtgatctatcgaggcgtcaatttcgccgagggcgtgatcgcttttctgattctggcaaagccaaaagaaaccttcctgcagagccctcccattagggaggccgtgaactacacagaaaacacttctagttactacgctacatcctacctggagtatgaaatcgagaactttggcgctcagcactctaccacactgttcaagattaacaataacacctttgtgctgctggatcgccctcatacaccacagttcctgtttcagctgaacgacactatccacctgcatcagcagctgagcaatactaccggaaaactgatttggacactggacgctaatatcaacgcagatattggcgagtgggccttctgggaaaataagaaaaacctgtccgagcagctgcggggagaggaactgagctttgaaacactgtccctgaatgaaactgaggacgatgacgccacctcaagccgaacaactaagggccggatctctgatcgggctaccagaaagtacagtgatctggtgccaaaagactctcccggcatggtgagtctgcacgtccctgaaggggagaccacactgccatcccagaactctactgagggccggagagtggacgtcaatacccaggagactatcaccgaaactaccgcaacaatcattggcactaacgggaataacatgcagatcagcaccattggcacagggctgtcctctagtcagattctgtcaagctcccctaccatggccccctcccctgagacacagacttctacaacttatacacccaagctgcctgtgatgaccacagaggaacccactaccccacccagaaacagtcctgggtcaacaactgaggcacccaccctgaccacacctgaaaatatcactaccgccgtgaaaacagtcctgcctcaggagtctactagtaacggactgatcaccagcacagtgactggaattctgggcagtctggggctgcgcaagcgatcaaggcgccaagtgaatactcgggctaccggcaaatgcaatccaaacctgcactactggaccgcacaggagcagcataacgccgctgggatcgcttggattccttacttcggaccaggcgcagaggggatctataccgaaggactgatgcataatcagaacgccctggtgtgtggcctgagacagctggcaaatgagacaactcaggccctgcagctgttcctgagagcaaccacagaactgaggacctatacaatcctgaaccggaaggccattgattttctgctgcgacgatggggcgggacctgcagaatcctgggaccagactgctgtattgagccccacgattggaccaagaacatcacagacaagatcaaccagatcattcatgatttcatcgacaacccactgcccaatcaggacaacgatgacaattggtggaccggatggcgacagtggattcccgcaggaattggaatcaccggaattattattgccattattgctctgctgtgtgtctgtaagctgctgtgttgataa

SEQ ID NO: 66 - DNA, 2049 bp, synthetic construct
  source 1..2049: mol_type = other DNA
atgaaaaccacttgtctgctgatctcactgattctgattcagggcgtcaaaacactgcccattctggaaattgcctctaacatccagccacagaacgtggactccgtctgttctgggaccctgcagaagacagaggatgtgcacctgatgggcttcaccctgagcgggcagaaggtcgcagactcacccctggaagccagcaaacgatgggcatttcgggccggagtgccccctaagaacgtcgagtacaccgaaggcgaggaagccaaaacatgctataatatctccgtgactgatcctagtggcaagtcactgctgctggacccacccaccaacattagggattaccctaagtgtaaaacaatccaccatattcagggccagaatccacacgctcaggggatcgcactgcatctgtggggagccttctttctgtacgacaggattgctagcaccacaatgtatcgcgggaaagtgttcaccgagggaaacatcgccgctatgattgtgaataagacagtccacaaaatgatcttttctcgccagggccaggggtaccgacatatgaacctgaccagtacaaataagtattggaccagctccaacggcactcagaccaatgacactgggtgcttcggaaccctgcaggagtacaacagtactaaaaatcagacctgtgctccatcaaagaaaccactgccactgcctaccgcacacccagaggtgaagctgacaagtacttcaaccgacgccacaaaactgaacactaccgaccccaatagtgacgatgaagatctgacaactagcggatccggctctggggagcaggaaccttataccacatccgatgcagccaccaagcagggcctgtctagtacaatgcctccaactccatctccccagcctagtactccccagcagggcgggaacaataccaaccattcccagggcgtggtcacagagccagggaagactaacactaccgcccagccctctatgccccctcacaatacaactaccatctccaccaacaatacatctaaacataacctgagcacaccttccgtgccaatccagaacgctactaactacaacactcagtctaccgcacccgagaatgaacagacttctgcccctagtaagacaactctgctgcccaccgagaaccctaccacagccaagtcaacaaatagcactaaatcccctactaccacagtgccaaacactaccaataagtacagtacctcaccaagccccacccctaactccacagcacagcacctggtctatttccggagaaaaagaaatatcctgtggagggagggcgacatgttcccttttctggatgggctgatcaacgctccaattgacttcgatccagtgcccaatacaaagactatctttgacgaatcaagctcctctggcgcctctgctgaggaagatcagcacgcctcacccaacattagcctgacactgtcctactttcctaaagtgaacgagaatactgcccatagcggggagaacgaaaatgactgcgatgctgagctgcggatctggagcgtccaggaagacgatctggctgcaggactgtcctggatcccattctttggacccggcattgagggactgtataccgccggcctgattaagaaccagaacaacctggtgtgcagactgaggcgcctggccaatcagaccgctaaatcactggaactgctgctgcgggtcacaactgaggaaagaacattcagcctgatcaaccgacatgctattgactttctgctggcacgctggggaggcacctgcaaggtgctgggaccagactgctgtatcggcattgaggatctgtctcgcaatatcagtgaacagatcgaccagattaagaaagatgagcagaaggaaggaaccggatggggactgggcggcaagtggtggaccagcgattggggcgtgctgacaaacctgggaatcctgctgctgctgtccatcgccgtcctgattgctctgtcctgtatttgtcggattttcactaagtatattgggtgataa